European Patent Application EP 4 516 306 A1, published March 5, 2025. Title: Therapeutic cancer vaccine using breast cancer cell adapted chimeric Zika virus. Applicant: SK bioscience Co., Ltd. Application KR. The sequence listing filed with the application follows.

SEQUENCE LISTING (41 sequences)

SEQ ID NO: 1 - DNA, 10862 bp, synthetic construct
  misc_feature 1..10862: note = backbone genome of YFV
  source 1..10862: mol_type = other DNA
agtaaatcctgtgtgctaattgaggtgcattggtctgcaaatcgagttgctaggcaataaacacatttggattaattttaatcgttcgttgagcgattagcagagaactgaccagaacatgtctggtcgtaaagctcagggaaaaaccctgggcgtcaatatggtacgacgaggagttcgctccttgtcaaacaaaataaaacaaaaaacaaaacaaattggaaacagacctggaccttcaagaggtgttcaaggatttatctttttctttttgttcaacattttgactggaaaaaagatcacagcccacctaaagaggttgtggaaaatgctggacccaagacaaggcttggctgttctaaggaaagtcaagagagtggtggccagtttgatgagaggattgtcctcaaggaaacgccgttcccatgatgttctgactgtgcaattcctaattttgggaatgctgttgatgacgggtggagtgaccttggtgcggaaaaacagatggttgctcctaaatgtgacatctgaggacctcgggaaaacattctctgtgggcacaggcaactgcacaacaaacattttggaagccaagtactggtgcccagactcaatggaatacaactgtcccaatctcagtccaagagaggagccagatgacattgattgctggtgctatggggtggaaaacgttagagtcgcatatggtaagtgtgactcagcaggcaggtctaggaggtcaagaagggccattgacttgcctacgcatgaaaaccatggtttgaagacccggcaagaaaaatggatgactggaagaatgggtgaaaggcaactccaaaagattgagagatggttcgtgaggaaccccttttttgcagtgacggctctgaccattgcctaccttgtgggaagcaacatgacgcaacgagtcgtgattgccctactggtcttggctgttggtccggcctactcagctcactgcattggaattactgacagggatttcattgagggggtgcatggaggaacttgggtttcagctaccctggagcaagacaagtgtgtcactgttatggcccctgacaagccttcattggacatctcactagagacagtagccattgatagacctgctgaggtgaggaaagtgtgttacaatgcagttctcactcatgtgaagattaatgacaagtgccccagcactggagaggcccacctagctgaagagaacgaaggggacaatgcgtgcaagcgcacttattctgatagaggctggggcaatggctgtggcctatttgggaaagggagcattgtggcatgcgccaaattcacttgtgccaaatccatgagtttgtttgaggttgatcagaccaaaattcagtatgtcatcagagcacaattgcatgtaggggccaagcaggaaaattggaataccgacattaagactctcaagtttgatgccctgtcaggctcccaggaagtcgagttcattgggtatggaaaagctacactggaatgccaggtgcaaactgcggtggactttggtaacagttacatcgctgagatggaaacagagagctggatagtggacagacagtgggcccaggacttgaccctgccatggcagagtggaagtggcggggtgtggagagagatgcatcatcttgtcgaatttgaacctccgcatgccgccactatcagagtactggccctgggaaaccaggaaggctccttgaaaacagctcttactggcgcaatgagggttacaaaggacacaaatgacaacaacctttacaaactacatggtggacatgtttcttgcagagtgaaattgtcagctttgacactcaaggggacatcctacaaaatatgcactgacaaaatgttttttgtcaagaacccaactgacactggccatggcactgttgtgatgcaggtgaaagtgtcaaaaggagccccctgcaggattccagtgatagtagctgatgatcttacagcggcaatcaataaaggcattttggttacagttaaccccatcgcctcaaccaatgatgatgaagtgctgattgaggtgaacccaccttttggagacagctacattatcgttgggagaggagattcacgtctcacttaccagtggcacaaagagggaagctcaataggaaagttgttcactcagaccatgaaaggcgtggaacgcctggccgtcatgggagacaccgcctgggatttcagctccgctggagggttcttcacttcggttgggaaaggaattcatacggtgtttggctctgcctttcaggggctatttggcggcttgaactggataacaaaggtcatcatgggggcggtacttatatgggttggcatcaacacaagaaacatgacaatgtccatgagcatgatcttggtaggagtgatcatgatgtttttgtctctaggagttggggcggatcaaggatgcgccatcaactttggcaagagagagctcaagtgcggagatggtatcttcatatttagagactctgatgactggctgaacaagtactcatactatccagaagatcctgtgaagcttgcatcaatagtgaaagcctcttttgaagaagggaagtgtggcctaaattcagttgactcccttgagcatgagatgtggagaagcagggcagatgagatcaatgccatttttgaggaaaacgaggtggacatttctgttgtcgtgcaggatccaaagaatgtttaccagagaggaactcatccattttccagaattcgggatggtctgcagtatggttggaagacttggggtaagaaccttgtgttctccccagggaggaagaatggaagcttcatcatagatggaaagtccaggaaagaatgcccgttttcaaaccgggtctggaattctttccagatagaggagtttgggacgggagtgttcaccacacgcgtgtacatggacgcagtctttgaatacaccatagactgcgatggatctatcttgggtgcagcggtgaacggaaaaaagagtgcccatggctctccaacattttggatgggaagtcatgaagtaaatgggacatggatgatccacaccttggaggcattagattacaaggagtgtgagtggccactgacacatacgattggaacatcagttgaagagagtgaaatgttcatgccgagatcaatcggaggcccagttagctctcacaatcatatccctggatacaaggttcagacgaacggaccttggatgcaggtaccactagaagtgaagagagaagcttgcccagggactagcgtgatcattgatggcaactgtgatggacggggaaaatcaaccagatccaccacggatagcgggaaagttattcctgaatggtgttgccgctcctgcacaatgccgcctgtgagcttccatggtagtgatgggtgttggtatcccatggaaattaggccaaggaaaacgcatgaaagccatctggtgcgctcctgggttacagctggagaaatacatgctgtcccttttggtttggtgagcatgatgatagcaatggaagtggtcctaaggaaaagacagggaccaaagcaaatgttggttggaggagtagtgctcttgggagcaatgctggtcgggcaagtaactctccttgatttgctgaaactcacagtggctgtgggattgcatttccatgagatgaacaatggaggagacgccatgtatatggcgttgattgctgccttttcaatcagaccagggctgctcatcggctttgggctcaggaccctatggagccctcgggaacgccttgtgctgaccctaggagcagccatggtggagattgccttgggtggcgtgatgggcggcctgtggaagtatctaaatgcagtttctctctgcatcctgacaataaatgctgttgcttctaggaaagcatcaaataccatcttgcccctcatggctctgttgacacctgtcactatggctgaggtgagacttgccgcaatgttcttttgtgccgtggttatcataggggtccttcaccagaatttcaaggacacctccatgcagaagactatacctctggtggccctcacactcacatcttacctgggcttgacacaaccttttttgggcctgtgtgcatttctggcaacccgcatatttgggcgaaggagtatcccagtgaatgaggcactcgcagcagctggtctagtgggagtgctggcaggactggcttttcaggagatggagaacttccttggtccgattgcagttggaggactcctgatgatgctggttagcgtggctgggagggtggatgggctagagctcaagaagcttggtgaagtttcatgggaagaggaggcggagatcagcgggagttccgcccgctatgatgtggcactcagtgaacaaggggagttcaagctgctttctgaagagaaagtgccatgggaccaggttgtgatgacctcgctggccttggttggggctgccctccatccatttgctcttctgctggtccttgctgggtggctgtttcatgtcaggggagctaggagaagtggggatgtcttgtgggatattcccactcctaagatcatcgaggaatgtgaacatctggaggatgggatttatggcatattccagtcaaccttcttgggggcctcccagcgaggagtgggagtggcacagggaggggtgttccacacaatgtggcatgtcacaagaggagctttccttgtcaggaatggcaagaagttgattccatcttgggcttcagtaaaggaagaccttgtcgcctatggtggctcatggaagttggaaggcagatgggatggagaggaagaggtccagttgatcgcggctgttccaggaaagaacgtggtcaacgtccagacaaaaccgagcttgttcaaagtgaggaatgggggagaaatcggggctgtcgctcttgactatccgagtggcacttcaggatctcctattgttaacaggaacggagaggtgattgggctgtacggcaatggcatccttgtcggtgacaactccttcgtgtccgccatatcccagactgaggtgaaggaagaaggaaaggaggagctccaagagatcccgacaatgctaaagaaaggaatgacaactgtccttgattttcatcctggagctgggaagacaagacgtttcctcccacagatcttggccgagtgcgcacggagacgcttgcgcactcttgtgttggcccccaccagggttgttctttctgaaatgaaggaggcttttcacggcctggacgtgaaattccacacacaggctttttccgctcacggcagcgggagagaagtcattgatgccatgtgccatgccaccctaacttacaggatgttggaaccaactagggttgttaactgggaagtgatcattatggatgaagcccattttttggatccagctagcatagccgctagaggttgggcagcgcacagagctagggcaaatgaaagtgcaacaatcttgatgacagccacaccgcctgggactagtgatgaatttccacattcaaatggtgaaatagaagatgttcaaacggacatacccagtgagccctggaacacagggcatgactggatcctagctgacaaaaggcccacggcatggttccttccatccatcagagctgcaaatgtcatggctgcctctttgcgtaaggctggaaagagtgtggtggtcctgaacaggaaaacctttgagagagaataccccacgataaagcagaagaaacctgactttatattggccactgacatagctgaaatgggagccaacctttgcgtggagcgagtgctggattgcaggacggcttttaagcctgtgcttgtggatgaagggaggaaggtggcaataaaagggccacttcgtatctccgcatcctctgctgctcaaaggagggggcgcattgggagaaatcccaacagagatggagactcatactactattctgagcctacaagtgaaaataatgcccaccacgtctgctggttggaggcctcaatgctcttggacaacatggaggtgaggggtggaatggtcgccccactctatggcgttgaaggaactaaaacaccagtttcccctggtgaaatgagactgagggatgaccagaggaaagtcttcagagaactagtgaggaattgtgacctgcccgtttggctttcgtggcaagtggccaaggctggtttgaagacgaatgatcgtaagtggtgttttgaaggccctgaggaacatgagatcttgaatgacagcggtgaaacagtgaagtgcagggctcctggaggagcaaagaagcctctgcgcccaaggtggtgtgatgaaagggtgtcatctgaccagagtgcgctgtctgaatttattaagtttgctgaaggtaggaggggagctgctgaagtgctagttgtgctgagtgaactccctgatttcctggctaaaaaaggtggagaggcaatggataccatcagtgtgttcctccactctgaggaaggctctagggcttaccgcaatgcactatcaatgatgcctgaggcaatgacaatagtcatgctgtttatactggctggactactgacatcgggaatggtcatctttttcatgtctcccaaaggcatcagtagaatgtctatggcgatgggcacaatggccggctgtggatatctcatgttccttggaggcgtcaaacccactcacatctcctatgtcatgctcatattctttgtcctgatggtggttgtgatccccgagccagggcaacaaaggtccatccaagacaaccaagtggcatacctcattattggcatcctgacgctggtttcagcggtggcagccaacgagctaggcatgctggagaaaaccaaagaggacctctttgggaagaagaacttaattccatctagtgcttcaccctggagttggccggatcttgacctgaagccaggagctgcctggacagtgtacgttggcattgttacaatgctctctccaatgttgcaccactggatcaaagtcgaatatggcaacctgtctctgtctggaatagcccagtcagcctcagtcctttctttcatggacaaggggataccattcatgaagatgaatatctcggtcataatgctgctggtcagtggctggaattcaataacagtgatgcctctgctctgtggcatagggtgcgccatgctccactggtctctcattttacctggaatcaaagcgcagcagtcaaagcttgcacagagaagggtgttccatggcgttgccgagaaccctgtggttgatgggaatccaacagttgacattgaggaagctcctgaaatgcctgccctttatgagaagaaactggctctatatctccttcttgctctcagcctagcttctgttgccatgtgcagaacgcccttttcattggctgaaggcattgtcctagcatcagctgccttagggccgctcatagagggaaacaccagccttctttggaatggacccatggctgtctccatgacaggagtcatgagggggaatcactatgcttttgtgggagtcatgtacaatctatggaagatgaaaactggacgccgggggagcgcgaatggaaaaactttgggtgaagtctggaagagggaactgaatctgttggacaagcgacagtttgagttgtataaaaggaccgacattgtggaggtggatcgtgatacggcacgcaggcatttggccgaagggaaggtggacaccggggtggcggtctccagggggaccgcaaagttaaggtggttccatgagcgtggctatgtcaagctggaaggtagggtgattgacctggggtgtggccgcggaggctggtgttactacgctgctgcgcaaaaggaagtgagtggggtcaaaggatttactcttggaagagacggccatgagaaacccatgaatgtgcaaagtctgggatggaacatcatcaccttcaaggacaaaactgatatccaccgcctagaaccagtgaaatgtgacacccttttgtgtgacattggagagtcatcatcgtcatcggtcacagagggggaaaggaccgtgagagttcttgatactgtagaaaaatggctggcttgtggggttgacaacttctgtgtgaaggtgttagctccatacatgccagatgttctcgagaaactggaattgctccaaaggaggtttggcggaacagtgatcaggaaccctctctccaggaattccactcatgaaatgtactacgtgtctggagcccgcagcaatgtcacatttactgtgaaccaaacatcccgcctcctgatgaggagaatgaggcgtccaactggaaaagtgaccctggaggctgacgtcatcctcccaattgggacacgcagtgttgagacagacaagggacccctggacaaagaggccatagaagaaagggttgagaggataaaatctgagtacatgacctcttggttttatgacaatgacaacccctacaggacctggcactactgtggctcctatgtcacaaaaacctcaggaagtgcggcgagcatggtaaatggtgttattaaaattctgacatatccatgggacaggatagaggaggtcacaagaatggcaatgactgacacaaccccttttggacagcaaagagtgtttaaagaaaaagttgacaccagagcaaaggatccaccagcgggaactaggaagatcatgaaagttgtcaacaggtggctgttccgccacctggccagagaaaagaaccccagactgtgcacaaaggaagaatttattgcaaaagtccgaagtcatgcagccattggagcttacctggaagaacaagaacagtggaagactgccaatgaggctgtccaagacccaaagttctgggaactggtggatgaagaaaggaagctgcaccaacaaggcaggtgtcggacttgtgtgtacaacatgatggggaaaagagagaagaagctgtcagagtttgggaaagcaaagggaagccgtgccatatggtatatgtggctgggagcgcggtatcttgagtttgaggccctgggattcctgaatgaggaccattgggcttccagggaaaactcaggaggaggagtggaaggcattggcttacaatacctaggatatgtgatcagagacctggctgcaatggatggtggtggattctacgcggatgacaccgctggatgggacacgcgcatcacagaggcagaccttgatgatgaacaggagatcttgaactacatgagcccacatcacaaaaaactggcacaagcagtgatggaaatgacatacaagaacaaagtggtgaaagtgttgagaccagccccaggagggaaagcctacatggatgtcataagtcgacgagaccagagaggatccgggcaggtagtgacttatgctctgaacaccatcaccaacttgaaagtccaattgatcagaatggcagaagcagagatggtgatacatcaccaacatgttcaagattgtgatgaatcagttctgaccaggctggaggcatggctcactgagcacggatgtgacagactgaagaggatggcggtgagtggagacgactgtgtggtccggcccatcgatgacaggttcggcctggccctgtcccatctcaacgccatgtccaaggttagaaaggacatatctgaatggcagccatcaaaagggtggaatgattgggagaatgtgcccttctgttcccaccacttccatgaactacagctgaaggatggcaggaggattgtggtgccttgccgagaacaggacgagctcattgggagaggaagggtgtctccaggaaacggctggatgatcaaggaaacagcttgcctcagcaaagcctatgccaacatgtggtcactgatgtattttcacaaaagggacatgaggctactgtcattggctgtttcctcagctgttcccacctcatgggttccacaaggacgcacaacatggtcgattcatgggaaaggggagtggatgaccacggaagacatgcttgaggtgtggaacagagtatggataaccaacaacccacacatgcaggacaagacaatggtgaaaaaatggagagatgtcccttatctaaccaagagacaagacaagctgtgcggatcactgattggaatgaccaatagggccacctgggcctcccacatccatttagtcatccatcgtatccgaacgctgattggacaggagaaatacactgactacctaacagtcatggacaggtattctgtggatgctgacctgcaactgggtgagcttatctgaaacaccatctaacaggaataaccgggatacaaaccacgggtggagaaccggactccccacaacctgaaaccgggatataaaccacggctggagaaccgggctccgcacttaaaatgaaacagaaaccgggataaaaactacggatggagaaccggactccacacattgagacagaagaagttgtcagcccagaaccccacacgagttttgccactgctaagctgtgaggcagtgcaggctgggacagccgacctccaggttgcgaaaaacctggtttctgggacctcccaccccagagtaaaaagaacggagcctccgctaccaccctcccacgtggtggtagaaagacggggtctagaggttagaggagaccctccagggaacaaatagtgggaccatattgacgccagggaaagaccggagtggttctctgcttttcctccagaggtctgtgagcacagtttgctcaagaataagcagacctttggatgacaaacacaaaaccact

SEQ ID NO: 2 - protein, 101 aa, synthetic construct
  REGION 1..101: note = Capsid protein of YFV
MSGRKAQGKTLGVNMVRRGVRSLSNKIKQKTKQIGNRPGPSRGVQGFIFFFLFNILTGKKITAHLKRLWKMLDPRQGLAVLRKVKRVVASLMRGLSSRKRR

SEQ ID NO: 3 - protein, 168 aa, synthetic construct
  REGION 1..168: note = prM protein of cZIKV
  TRANSMEM 94..168: note = prM membrain protein
AEVTRRGSAYYMYLDRNDAGEAISFPTTLGMNKCYIQIMDLGHMCDATMSYECPMLDEGVEPDDVDCWCNTTSTWVVYGTCHHKKGEARRSRRAVTLPSHSTRKLQTRSQTWLESREYTKHLIRVENWIFRNPGFALAAAAIAWLLGSSTSQKVIYLVMILLIAPAYS

SEQ ID NO: 4 - protein, 504 aa, synthetic construct
  REGION 1..504: note = Envelop protein of cZIKV
  TRANSMEM 460..504: note = Envelop membrain protein
IRCIGVSNRDFVEGMSGGTWVDVVLEHGGCVTVMAQDKPTVDIELVTTTVSNMAEVRSYCYEASISDMASDSRCPTQGEAYLDKQSDTQYVCKRTLVDRGWGNGCGLFGKGSLVTCAKFACSKKMTGKSIQPENLEYRIMLSVHGSQHSGMIVNDTGHETDENRAKVEITPNSPRAEATLGGFGSLGLDCEPRTGLDFSDLYYLTMNNKHWLVHKEWFHDIPLPWHAGADTGTPHWNNKEALVEFKDAHAKRQTVVVLGSQEGAVHTALAGALEAEMDGAKGRLSSGHLKCRLKMDKLRLKGVSYSLCTAAFTFTKIPAETLHGTVTVEVQYAGTDGPCKVPAQMAVDMQTLTPVGRLITANPVITESTENSKMMLELDPPFGDSYIVIGVGEKKITHHWHRSGSTIGKAFEATVRGAKRMAVLGDTAWDFGSVGGALNSLGKGIHQIFGAAFKSLFGGMSWFSQILIGTLLMWLGLNTKNGSISLMCLALGGVLIFLSTAVSA

SEQ ID NO: 5 - protein, 2633 aa, synthetic construct
  REGION 1..2633: note = non-structure protein of YFV
DQGCAINFGKRELKCGDGIFIFRDSDDWLNKYSYYPEDPVKLASIVKASFEEGKCGLNSVDSLEHEMWRSRADEINAIFEENEVDISVVVQDPKNVYQRGTHPFSRIRDGLQYGWKTWGKNLVFSPGRKNGSFIIDGKSRKECPFSNRVWNSFQIEEFGTGVFTTRVYMDAVFEYTIDCDGSILGAAVNGKKSAHGSPTFWMGSHEVNGTWMIHTLEALDYKECEWPLTHTIGTSVEESEMFMPRSIGGPVSSHNHIPGYKVQTNGPWMQVPLEVKREACPGTSVIIDGNCDGRGKSTRSTTDSGKVIPEWCCRSCTMPPVSFHGSDGCWYPMEIRPRKTHESHLVRSWVTAGEIHAVPFGLVSMMIAMEVVLRKRQGPKQMLVGGVVLLGAMLVGQVTLLDLLKLTVAVGLHFHEMNNGGDAMYMALIAAFSIRPGLLIGFGLRTLWSPRERLVLTLGAAMVEIALGGVMGGLWKYLNAVSLCILTINAVASRKASNTILPLMALLTPVTMAEVRLAAMFFCAVVIIGVLHQNFKDTSMQKTIPLVALTLTSYLGLTQPFLGLCAFLATRIFGRRSIPVNEALAAAGLVGVLAGLAFQEMENFLGPIAVGGLLMMLVSVAGRVDGLELKKLGEVSWEEEAEISGSSARYDVALSEQGEFKLLSEEKVPWDQVVMTSLALVGAALHPFALLLVLAGWLFHVRGARRSGDVLWDIPTPKIIEECEHLEDGIYGIFQSTFLGASQRGVGVAQGGVFHTMWHVTRGAFLVRNGKKLIPSWASVKEDLVAYGGSWKLEGRWDGEEEVQLIAAVPGKNVVNVQTKPSLFKVRNGGEIGAVALDYPSGTSGSPIVNRNGEVIGLYGNGILVGDNSFVSAISQTEVKEEGKEELQEIPTMLKKGMTTVLDFHPGAGKTRRFLPQILAECARRRLRTLVLAPTRVVLSEMKEAFHGLDVKFHTQAFSAHGSGREVIDAMCHATLTYRMLEPTRVVNWEVIIMDEAHFLDPASIAARGWAAHRARANESATILMTATPPGTSDEFPHSNGEIEDVQTDIPSEPWNTGHDWILADKRPTAWFLPSIRAANVMAASLRKAGKSVVVLNRKTFEREYPTIKQKKPDFILATDIAEMGANLCVERVLDCRTAFKPVLVDEGRKVAIKGPLRISASSAAQRRGRIGRNPNRDGDSYYYSEPTSENNAHHVCWLEASMLLDNMEVRGGMVAPLYGVEGTKTPVSPGEMRLRDDQRKVFRELVRNCDLPVWLSWQVAKAGLKTNDRKWCFEGPEEHEILNDSGETVKCRAPGGAKKPLRPRWCDERVSSDQSALSEFIKFAEGRRGAAEVLVVLSELPDFLAKKGGEAMDTISVFLHSEEGSRAYRNALSMMPEAMTIVMLFILAGLLTSGMVIFFMSPKGISRMSMAMGTMAGCGYLMFLGGVKPTHISYVMLIFFVLMVVVIPEPGQQRSIQDNQVAYLIIGILTLVSAVAANELGMLEKTKEDLFGKKNLIPSSASPWSWPDLDLKPGAAWTVYVGIVTMLSPMLHHWIKVEYGNLSLSGIAQSASVLSFMDKGIPFMKMNISVIMLLVSGWNSITVMPLLCGIGCAMLHWSLILPGIKAQQSKLAQRRVFHGVAENPVVDGNPTVDIEEAPEMPALYEKKLALYLLLALSLASVAMCRTPFSLAEGIVLASAALGPLIEGNTSLLWNGPMAVSMTGVMRGNHYAFVGVMYNLWKMKTGRRGSANGKTLGEVWKRELNLLDKRQFELYKRTDIVEVDRDTARRHLAEGKVDTGVAVSRGTAKLRWFHERGYVKLEGRVIDLGCGRGGWCYYAAAQKEVSGVKGFTLGRDGHEKPMNVQSLGWNIITFKDKTDIHRLEPVKCDTLLCDIGESSSSSVTEGERTVRVLDTVEKWLACGVDNFCVKVLAPYMPDVLEKLELLQRRFGGTVIRNPLSRNSTHEMYYVSGARSNVTFTVNQTSRLLMRRMRRPTGKVTLEADVILPIGTRSVETDKGPLDKEAIEERVERIKSEYMTSWFYDNDNPYRTWHYCGSYVTKTSGSAASMVNGVIKILTYPWDRIEEVTRMAMTDTTPFGQQRVFKEKVDTRAKDPPAGTRKIMKVVNRWLFRHLAREKNPRLCTKEEFIAKVRSHAAIGAYLEEQEQWKTANEAVQDPKFWELVDEERKLHQQGRCRTCVYNMMGKREKKLSEFGKAKGSRAIWYMWLGARYLEFEALGFLNEDHWASRENSGGGVEGIGLQYLGYVIRDLAAMDGGGFYADDTAGWDTRITEADLDDEQEILNYMSPHHKKLAQAVMEMTYKNKVVKVLRPAPGGKAYMDVISRRDQRGSGQVVTYALNTITNLKVQLIRMAEAEMVIHHQHVQDCDESVLTRLEAWLTEHGCDRLKRMAVSGDDCVVRPIDDRFGLALSHLNAMSKVRKDISEWQPSKGWNDWENVPFCSHHFHELQLKDGRRIVVPCREQDELIGRGRVSPGNGWMIKETACLSKAYANMWSLMYFHKRDMRLLSLAVSSAVPTSWVPQGRTTWSIHGKGEWMTTEDMLEVWNRVWITNNPHMQDKTMVKKWRDVPYLTKRQDKLCGSLIGMTNRATWASHIHLVIHRIRTLIGQEKYTDYLTVMDRYSVDADLQLGELI

SEQ ID NO: 6 - protein, 20 aa, synthetic construct
  REGION 1..20: note = Signal peptide sequence present upstream of prM protein of cZIKV
SHDVLTVQFLILGMLLMTGG

SEQ ID NO: 7 - protein, 3426 aa, synthetic construct
  REGION 1..3426: note = cZIKV sequence in which ZIKV was introduced into YFV (sequence before mutation according to subculture)
MSGRKAQGKTLGVNMVRRGVRSLSNKIKQKTKQIGNRPGPSRGVQGFIFFFLFNILTGKKITAHLKRLWKMLDPRQGLAVLRKVKRVVASLMRGLSSRKRRSHDVLTVQFLILGMLLMTGGAEVTRRGSAYYMYLDRNDAGEAISFPTTLGMNKCYIQIMDLGHMCDATMSYECPMLDEGVEPDDVDCWCNTTSTWVVYGTCHHKKGEARRSRRAVTLPSHSTRKLQTRSQTWLESREYTKHLIRVENWIFRNPGFALAAAAIAWLLGSSTSQKVIYLVMILLIAPAYSIRCIGVSNRDFVEGMSGGTWVDVVLEHGGCVTVMAQDKPTVDIELVTTTVSNMAEVRSYCYEASISDMASDSRCPTQGEAYLDKQSDTQYVCKRTLVDRGWGNGCGLFGKGSLVTCAKFACSKKMTGKSIQPENLEYRIMLSVHGSQHSGMIVNDTGHETDENRAKVEITPNSPRAEATLGGFGSLGLDCEPRTGLDFSDLYYLTMNNKHWLVHKEWFHDIPLPWHAGADTGTPHWNNKEALVEFKDAHAKRQTVVVLGSQEGAVHTALAGALEAEMDGAKGRLSSGHLKCRLKMDKLRLKGVSYSLCTAAFTFTKIPAETLHGTVTVEVQYAGTDGPCKVPAQMAVDMQTLTPVGRLITANPVITESTENSKMMLELDPPFGDSYIVIGVGEKKITHHWHRSGSTIGKAFEATVRGAKRMAVLGDTAWDFGSVGGALNSLGKGIHQIFGAAFKSLFGGMSWFSQILIGTLLMWLGLNTKNGSISLMCLALGGVLIFLSTAVSADQGCAINFGKRELKCGDGIFIFRDSDDWLNKYSYYPEDPVKLASIVKASFEEGKCGLNSVDSLEHEMWRSRADEINAIFEENEVDISVVVQDPKNVYQRGTHPFSRIRDGLQYGWKTWGKNLVFSPGRKNGSFIIDGKSRKECPFSNRVWNSFQIEEFGTGVFTTRVYMDAVFEYTIDCDGSILGAAVNGKKSAHGSPTFWMGSHEVNGTWMIHTLEALDYKECEWPLTHTIGTSVEESEMFMPRSIGGPVSSHNHIPGYKVQTNGPWMQVPLEVKREACPGTSVIIDGNCDGRGKSTRSTTDSGKVIPEWCCRSCTMPPVSFHGSDGCWYPMEIRPRKTHESHLVRSWVTAGEIHAVPFGLVSMMIAMEVVLRKRQGPKQMLVGGVVLLGAMLVGQVTLLDLLKLTVAVGLHFHEMNNGGDAMYMALIAAFSIRPGLLIGFGLRTLWSPRERLVLTLGAAMVEIALGGVMGGLWKYLNAVSLCILTINAVASRKASNTILPLMALLTPVTMAEVRLAAMFFCAVVIIGVLHQNFKDTSMQKTIPLVALTLTSYLGLTQPFLGLCAFLATRIFGRRSIPVNEALAAAGLVGVLAGLAFQEMENFLGPIAVGGLLMMLVSVAGRVDGLELKKLGEVSWEEEAEISGSSARYDVALSEQGEFKLLSEEKVPWDQVVMTSLALVGAALHPFALLLVLAGWLFHVRGARRSGDVLWDIPTPKIIEECEHLEDGIYGIFQSTFLGASQRGVGVAQGGVFHTMWHVTRGAFLVRNGKKLIPSWASVKEDLVAYGGSWKLEGRWDGEEEVQLIAAVPGKNVVNVQTKPSLFKVRNGGEIGAVALDYPSGTSGSPIVNRNGEVIGLYGNGILVGDNSFVSAISQTEVKEEGKEELQEIPTMLKKGMTTVLDFHPGAGKTRRFLPQILAECARRRLRTLVLAPTRVVLSEMKEAFHGLDVKFHTQAFSAHGSGREVIDAMCHATLTYRMLEPTRVVNWEVIIMDEAHFLDPASIAARGWAAHRARANESATILMTATPPGTSDEFPHSNGEIEDVQTDIPSEPWNTGHDWILADKRPTAWFLPSIRAANVMAASLRKAGKSVVVLNRKTFEREYPTIKQKKPDFILATDIAEMGANLCVERVLDCRTAFKPVLVDEGRKVAIKGPLRISASSAAQRRGRIGRNPNRDGDSYYYSEPTSENNAHHVCWLEASMLLDNMEVRGGMVAPLYGVEGTKTPVSPGEMRLRDDQRKVFRELVRNCDLPVWLSWQVAKAGLKTNDRKWCFEGPEEHEILNDSGETVKCRAPGGAKKPLRPRWCDERVSSDQSALSEFIKFAEGRRGAAEVLVVLSELPDFLAKKGGEAMDTISVFLHSEEGSRAYRNALSMMPEAMTIVMLFILAGLLTSGMVIFFMSPKGISRMSMAMGTMAGCGYLMFLGGVKPTHISYVMLIFFVLMVVVIPEPGQQRSIQDNQVAYLIIGILTLVSAVAANELGMLEKTKEDLFGKKNLIPSSASPWSWPDLDLKPGAAWTVYVGIVTMLSPMLHHWIKVEYGNLSLSGIAQSASVLSFMDKGIPFMKMNISVIMLLVSGWNSITVMPLLCGIGCAMLHWSLILPGIKAQQSKLAQRRVFHGVAENPVVDGNPTVDIEEAPEMPALYEKKLALYLLLALSLASVAMCRTPFSLAEGIVLASAALGPLIEGNTSLLWNGPMAVSMTGVMRGNHYAFVGVMYNLWKMKTGRRGSANGKTLGEVWKRELNLLDKRQFELYKRTDIVEVDRDTARRHLAEGKVDTGVAVSRGTAKLRWFHERGYVKLEGRVIDLGCGRGGWCYYAAAQKEVSGVKGFTLGRDGHEKPMNVQSLGWNIITFKDKTDIHRLEPVKCDTLLCDIGESSSSSVTEGERTVRVLDTVEKWLACGVDNFCVKVLAPYMPDVLEKLELLQRRFGGTVIRNPLSRNSTHEMYYVSGARSNVTFTVNQTSRLLMRRMRRPTGKVTLEADVILPIGTRSVETDKGPLDKEAIEERVERIKSEYMTSWFYDNDNPYRTWHYCGSYVTKTSGSAASMVNGVIKILTYPWDRIEEVTRMAMTDTTPFGQQRVFKEKVDTRAKDPPAGTRKIMKVVNRWLFRHLAREKNPRLCTKEEFIAKVRSHAAIGAYLEEQEQWKTANEAVQDPKFWELVDEERKLHQQGRCRTCVYNMMGKREKKLSEFGKAKGSRAIWYMWLGARYLEFEALGFLNEDHWASRENSGGGVEGIGLQYLGYVIRDLAAMDGGGFYADDTAGWDTRITEADLDDEQEILNYMSPHHKKLAQAVMEMTYKNKVVKVLRPAPGGKAYMDVISRRDQRGSGQVVTYALNTITNLKVQLIRMAEAEMVIHHQHVQDCDESVLTRLEAWLTEHGCDRLKRMAVSGDDCVVRPIDDRFGLALSHLNAMSKVRKDISEWQPSKGWNDWENVPFCSHHFHELQLKDGRRIVVPCREQDELIGRGRVSPGNGWMIKETACLSKAYANMWSLMYFHKRDMRLLSLAVSSAVPTSWVPQGRTTWSIHGKGEWMTTEDMLEVWNRVWITNNPHMQDKTMVKKWRDVPYLTKRQDKLCGSLIGMTNRATWASHIHLVIHRIRTLIGQEKYTDYLTVMDRYSVDADLQLGELI

SEQ ID NO: 8 - protein, 3426 aa, synthetic construct
  REGION 1..3426: note = Virus Bx61 amino acid full-length sequence that has been subcultured
MSGRKAQGKTLGVNMVRRGVRSLSNKIKQETKQIGNRPGPSRGVQGFIFFFLFNILTGKRITAHLKRLWKMLDPRQGLAVLRKVKRVVASLMRGLSSRKRRSHDVLTVQFLILGMLLMTGGVEVTRRGSAYYMYLDRNDAGEAISFPTTLGMNKCYIQIMDLGHMCDATMSYECPMLDEGVEPDDVDCWCNTTSTWVVYGTCHHKKGEARRSRRAVTLPSHSTRKLRTRSQTWLESREYTKHLIRVENWIFRNPGFALAAAAIAWLLGSSTSQKVIYLVMILLIAPAYSIRCIGVSNRDFVEGMSGGTWVDVVLEHGGCVTVMAQDKPTVDIELVTTTVSNMAEVRSYCYEASISDMASDSRCPTQGEAYLDKQSDTQYVCKRTLVDRGWGNGCGLFGKGSLVTCAKFACSKKMTGKSIQPENLEYQIMLSVHGSQHSGMIVNDTGHETDENRAKVEITPNSPRAEATLGGFGSLGLDCEPRTGLDFSDLYYLTMNKKHWLVHKEWFHDIPLPWHAGADTGTPHWNNKEALVEFKDAHAKRQTVVVLGSQEGAVHTALAGALEAEMDGAKGRLSSGHLKCRLKMDKLRLKGVSYSLCTAAFTFTKIPTETLHGTVTVEVQYAGTDGPCKVPAQMAVDMQTLTPVGRLITANPVITEITENSKMMLELDPPFGDSYIVIGVGEKKITHHWYRSGSTIGKAFEATVRGAKRMAVLGDTAWDFGSVGGALNSLGKGIHQIFGAAFKSLFGGMSWFSQILIGTLLMWLGLNTKNGSISLMCLALGGVLIFLSTAVSADQGCAINFGKRELKCGDGIFIFRDSDDWLNKYSYYPEDPVKLASIVKASFEEGKCGLNSVDSLEHEMWRSRADEINAIFEENEVDISVVVQDPKNVYQRGTHPFSRIRDGLQYGWKTWGKNLVFSPGRKNGSFIIDGKSRKECPFSNRVWNSFQIEEFGTGVFTTRVYMDAVFEYTIDCDGSILGAAVNGKKSAHGSPTFWMGSHEVNGTWMIHTLEALDYKECEWPLTHTIGTSVEESEMFMPRSIGGPVSSHNHIPGYKVQTNGPWMQVPLEVKREACPGTSVIIDGNCDGRGKSTRSTTDSGKVIPEWCCRSCTMPPVSFHGSDGCWYPMEIRPRKTHESHLVRSWVTAGEIHAVPFGLVSMMIAMEVVLRKRQGPKQMLVGGVVLLGAMLVGQVTLLDLLKLTVAVGLHFHEMNNGGDAMYMALIAAFSIRPGLLIGFGLRTLWSPRERLVLTLGAAMVEIALGGVMGGLWKYLNAVSLCILTINAVASRKASNTILPLMALLTPVTMAEVRLAAMFFCAVVIIGVLHQNFKDTSMQKTIPLVALTLTSYLGLTQPFLGLCAFLATRIFGRRSIPVNEALAAAGLVGVLAGLAFQEMENFLGPIAVGGLLMMLVSVAGRVDGLELKKLGEVSWEEEAEISGSSARYDVALSEQGEFKLLSEEKVPWNQVVMTSLALVGAALHPFALLLVLAGWLFHVRGARRSGDVLWDIPTPKIIEECEHLEDGIYGIFQSTFLGASQRGVGVAQGGVFHTMWHVTRGAFLVRNGKKLIPSWASVKEDLVAYGGSWKLEGRWDGEEEVQLIAAVPGKNVVNVQTKPSLFKVRNGGEIGAVALDYPSGTSGSPIVNRNGEVIGLYGNGILVGDNSFVSAISQTEVKEEGKEELQEIPTMLKKGMTTVLDFHPGAGKTRRFLPQILAECARRRLRTLVLAPTRVVLSEMKEAFHGLDVKFHTQAFSAHGSGREVIDAMCHATLTYRMLEPTRVVNWEVIIMDEAHFLDPASIAARGWAAHRARANESATILMTATPPGTSDEFPHSNGEIEDVQTDMPSEPWNTGHDWILADKRPTAWFLPSIRAANVMAASLRKAGKSVVVLNRKTFEREYPTIKQKKPDFILATDIAEMGANLCVERVLDCRTAFKPVLVDEGRKVAIKGPLRISASSAAQRRGRIGRNPNRDGDSYYYSEPTSENNAHHVCWLEASMLLDNMEVRGGMVAPLYGVEGTKTPVSPGEMRLRDDQRKVFRELVRNCDLPVWLSWHVAKAGLKTNDRKWCFEGPEEHEILNDSGETVKCRAPGGAKKPLRPRWCDERVSSDHSALSEFIKFAEGRRGAAEVLVVLSELPDFLVKKGGEAMDTINVFLHSEEGSRAYRNALSMMPEAMTIVMLFILAGLLTSGMVIFFMSPKGISRMSMAMGTMAGCGYLMFLGGVKPTHISYVMLIFFVLMVVVIPEPGQQRSIQDNQVAYLIIGILTLVSAVAANELGMLEKTKEDLFGKKNLIPSSASPWSWPDLDLKPGAAWTVYVGIVTMLSPMLHHWIKVEYGNLSLSGIAQSASVLSLMDKGIPFMKMNISVIMLLVSGWNSITVMPLLCGIGCAMLHWSLILPGIKAQQSRLAQRRVFHGVAKNPVVDGNPTVDIEEAPEMPALYEKKLALYLLLALSLASVAMCRTSFSLAEGIVLASAALGPLIEGNTSLLWNGPMAVSMTGVMRGNHYAFVGVMYNLWKMKTGRRGSANGKTLGEVWKRELNLLDKRQFELYKRTDIVEVDRDTARRHLAEGKVDTGVAVSRGTAKLRWFHERGYVKLEGRVIDLGCGRGGWCYYAAAQKEVSGVKGFTLGRDGHEKPMNVQSLGWNIITFKDKTDIHRLEPVKCDTLLCDIGESSSSSVTEGERTVRVLDTVEKWLACGVDNFCVKVLAPYMPDVLEKLELLQRRFGGTVIRNPLSRNSTHEMYYVSGARSNVTFTVNQTSRLLMRRMRRPTGKVTLEADVILPIGTRSVETDKGPLDKEAIEERVERIKSEYMTSWFYDNDNPYRTWHYCGSYVTKTSGSAASMVNGVIKILTYPWDRIEEVTRMAMTDTTPFGQQRVFKEKVDTRAKDPPAGTRKIMKVVNRWLFRHLAREKNPRLCTKEEFIAKVRSHAAIGAYLEEQEQWKTANEAVQDPKFWELVDEERKLHQQGRCRTCVYNMMGKREKKLSEFGKAKGSRAIWYMWLGARYLEFEALGFLNEDHWASRENSGGGVEGIGLQYLGYVIRDLAAMDGGGFYADDTAGWDTRITEADLDDEQEILIYMSPHHKKLAQAVMEMTYKNKVVKVLRPAPGGKAYMDVISRRDQRGSGQVVTYALNTITNLKVQLIRMAEAEMVIHHQHVQDCDESVLTRLEAWLTEHGCDRLKRMAVSGDDCVVRPIDDRFGLALSHLNAMSKVRKDISEWQPSKGWNDWENVPFCSHHFHELQLKDGRRIVVPCREQDELIGRGRVSPGNGWMIKETACLSKAYANMWSLMYFHKRDMRLLSLAVSSAVPTSWVPQGRTTWSIHGKGEWMTTEDMLEVWNRVWITNNPHMQDKTMVKKWRDVPYLTKRQDKLCGSLIGMTNRATWASHIHLVIHRIRTLIGQEKYTDYLTVMDRYSVDADLQLGELI

SEQ ID NO: 9 - DNA, 10787 bp, synthetic construct
  misc_feature 1..10787: note = Virus Bx61 nucleotide full-length sequence that has been subcultured
  source 1..10787: mol_type = other DNA
atgtctggtcgtaaagctcagggaaaaaccctgggcgtcaatatggtacgacgaggagttcgctccttgtcaaacaaaataaaacaagaaacaaaacaaattggaaacagacctggaccttcaagaggtgttcaaggatttatctttttctttttgttcaacattttgactggaaaaaggatcacagcccacctaaagaggttgtggaaaatgctggacccaagacaaggcttggctgttctaaggaaagtcaagagagtggtggccagtttgatgagaggattgtcctcaaggaaacgccgttcccatgatgttctgactgtgcaattcctaattttgggaatgctgttgatgacgggtggagtggaggtcactagacgtgggagtgcatactatatgtacttggacagaaacgatgctggggaggccatatcttttccaaccacattggggatgaataagtgttatatacagatcatggatcttggacacatgtgtgatgccaccatgagctatgaatgccctatgctggatgagggggtggaaccagatgacgtcgattgttggtgcaacacgacgtcaacttgggttgtgtacggaacctgccatcacaaaaaaggtgaagcacgtagatctagaagagctgtgacgctcccctcccattccactaggaagctgcgaacgcggtcgcaaacctggttggaatcaagagaatacacaaagcacttgattagagtcgaaattggatattcaggaaccctggcttcgcgttagcagcagctgccatcgcttggcttttgggaagctcaacgagccaaaaagtcatatacttggtcatgatactgctgattgccccggcatacagcatcaggtgcataggagtcagcaatagggactttgtggaaggtatgtcaggtgggacttgggttgatgttgtcttggaacatggaggttgtgtcaccgtaatggcacaggacaaaccgactgtcgacatagagctggttacaacaacagtcagcaacatggcggaggtaagatcctactgctatgaggcatcaatatcagacatggcttcggacagccgctgcccaacacaaggtgaagcctaccttgacaagcaatcagacactcaatatgtctgcaaaagaacgttagtggacagaggctggggaaatggatgtggactttttggcaaagggagcctggtgacatgcgctaaatttgcatgctccaagaaaatgaccgggaagagcatccagccagagaatctggagtaccagataatgctgtcagttcatggctcccagcacagtgggatgatcgttaatgacacaggacatgaaactgatgagaatagagcgaaagttgagataacgcccaattcaccaagagccgaagccaccctggggggttttggaagcctaggacttgattgtgaaccgaggacaggccttgacttttcagatttgtattacttgactatgaataaaaagcactggttggttcacaaggagtggttccacgacattccattaccttggcacgctggggcagacaccggaactccacactggaacaacaaagaagcactggtagagttcaaggacgcacatgccaaaaggcaaactgtcgtggttctagggagtcaagaaggagcagttcacacggcccttgctggagctctggaggctgagatggatggtgcaaagggaaggctgtcctctggccacttgaaatgtcgcctgaaaatggataaacttagattgaagggcgtgtcatactccttgtgtactgcagcgttcacattcaccaagatcccgactgaaacactgcacgggacagtcacagtggaggtacagtacgcagggacagatggaccttgcaaggttccagctcagatggcggtggacatgcaaactctgaccccagttgggaggttgataaccgctaaccccgtaatcactgaaatcactgagaactctaagatgatgctggaacttgatccaccatttggggactcttacattgtcataggagtcggggagaagaagatcacccaccactggtacaggagtggcagcaccattggaaaagcatttgaagccactgtgagaggtgccaagagaatggcagtcttgggagacacagcctgggactttggatcagttggaggcgctctcaactcattgggcaagggcatccatcaaatttttggagcagctttcaaatcattgtttggaggaatgtcctggttctcacaaattctcattggaacgttgctgatgtggttgggtctgaacacaaagaatggatctatttcccttatgtgcttggccttagggggggtgttgatcttcttatccacagccgtctctgctgatcaaggatgcgccatcaactttggcaagagagagctcaagtgcggagatggtatcttcatatttagagactctgatgactggctgaacaagtactcatactatccagaagatcctgtgaagcttgcatcaatagtgaaagcctcttttgaagaagggaagtgtggcctaaattcagttgactcccttgagcatgagatgtggagaagcagggcagatgagatcaatgccatttttgaggaaaacgaggtggacatttctgttgtcgtgcaggatccaaagaatgtttaccagagaggaactcatccattttccagaattcgggatggtctgcagtatggttggaagacttggggtaagaaccttgtgttctccccagggaggaagaatggaagcttcatcatagatggaaagtccaggaaagaatgcccgttttcaaaccgggtctggaattctttccagatagaggagtttgggacgggagtgttcaccacacgcgtgtacatggacgcagtctttgaatacaccatagactgcgatggatctatcttgggtgcagcggtgaacggaaaaaagagtgcccatggctctccaacattttggatgggaagtcatgaagtaaatgggacatggatgatccacaccttggaggcattagattacaaggagtgtgagtggccactgacacatacgattggaacatcagttgaagagagtgaaatgttcatgccaagatcaatcggaggcccagttagctctcacaatcatatccctggatacaaggttcagacgaacggaccttggatgcaggtgccactagaagtgaagagagaagcttgcccagggactagcgtgatcattgatggcaactgtgatggacggggaaaatcaaccagatccaccacggatagcgggaaagttattcctgaatggtgttgccgctcctgcacaatgccgcctgtgagcttccatggtagtgatgggtgttggtatcccatggaaattaggccaaggaaaacgcatgaaagccatctggtgcgctcttgggttacagctggagaaatacatgctgtcccttttggtttggtgagcatgatgatagcaatggaagtggtcctaaggaaaagacagggaccaaagcaaatgttggttggaggagtagtgctcttgggagcaatgctggtcgggcaagtaactctccttgatttgctgaaactcacagtggctgtgggattgcatttccatgagatgaacaatggaggagacgccatgtatatggcgttgattgctgccttttcaatcagaccagggctgctcatcggctttgggctcaggaccctatggagccctcgggaacgccttgtgctgaccctaggagcagccatggtggagattgccttgggtggcgtgatgggcggcctgtggaagtatctaaatgcagtttctctctgcatcctgacaataaatgctgttgcttctaggaaagcatcaaataccatcttgcccctcatggctctgttgacacctgtcactatggctgaggtgagacttgccgcaatgttcttttgtgccgtggttatcataggggtccttcaccagaatttcaaggacacctccatgcagaagactatacctctggtggccctcacactcacatcttacctgggcttaacacaaccttttttgggcctgtgtgcatttctggcaacccgcatatttgggcgaaggagtatcccagtgaatgaggcactcgcagcagctggtctagtgggagtgctggcaggactggcttttcaggagatggagaacttccttggtccgattgcagttggaggactcctgatgatgctggttagcgtggctgggagggtggatgggctagagctcaagaagcttggtgaagtttcatgggaagaggaggcggagatcagcgggagttccgcccgctatgatgtggcactcagtgaacaaggggagttcaagctgctttctgaagagaaagtgccatggaaccaggttgtgatgacctcgctggccttggttggggctgccctccatccatttgctcttctgctggtccttgctgggtggctgtttcatgtcaggggagctaggagaagtggggatgtcttgtgggatattcccactcctaagatcatcgaggaatgtgaacatctggaggatgggatttatggcatattccagtcaaccttcttgggggcctcccagcgaggagtgggagtggcacagggaggggtgttccacacaatgtggcatgtcacaagaggagctttccttgtcaggaatggcaagaagttgattccatcttgggcttcagtaaaggaagaccttgtcgcctatggtggctcatggaagttggaaggcagatgggatggagaggaagaggtccagttgatcgcggctgttccaggaaagaacgtggtcaacgtccagacaaaaccgagcttgttcaaagtgaggaatgggggagaaatcggggctgtcgctcttgactatccgagtggcacttcaggatctcctattgttaacaggaacggagaggtgattgggctgtacggcaatggcatccttgtcggtgacaactccttcgtgtccgccatatcccagactgaggtgaaggaagaaggaaaggaggagctccaagagatcccgacaatgttaaagaaaggaatgacaactgtccttgattttcatcctggagctgggaagacaagacgtttcctcccacagatcttggccgagtgcgcacggagacgcttgcgcactcttgtgttggcccccaccagggttgttctttctgaaatgaaggaggcttttcacggcctggacgtgaaattccacacacaggctttttccgctcacggcagcgggagagaagtcattgatgccatgtgccatgccaccctaacttacaggatgttggaaccaactagggttgttaactgggaagtgatcattatggatgaagcccattttttggatccagctagcatagccgctagaggttgggcagcgcacagagctagggcaaatgaaagtgcaacaatcttgatgacagccacaccgcctgggactagtgatgaatttccacattcaaatggtgaaatagaagatgttcaaacggacatgcccagtgagccctggaacacagggcatgactggatcctagctgacaaaaggcccacggcatggttccttccatccatcagagctgcaaatgtcatggctgcctctttgcgtaaggctggaaagagtgtggtggtcctgaacaggaaaacctttgagagagaataccccacgataaagcagaagaaacctgactttatattggccactgacatagctgaaatgggagccaacctctgcgtggagcgagtgctggattgcaggacggcttttaagcctgtgcttgtggatgaagggaggaaggtggcaataaaagggccacttcgtatctccgcatcctctgctgctcagaggagggggcgcattgggagaaatcccaacagagatggagactcatactactattctgagcctacaagtgaaaataatgcccaccacgtctgttggttggaggcctcaatgctcttggacaacatggaggtgaggggtggaatggtcgccccactctatggcgttgaaggaactaaaacaccagtttcccctggtgaaatgagactgagggatgaccagaggaaagtcttcagagaactagtgaggaattgtgacctgcccgtttggctttcgtggcacgtggccaaagctggtttgaagacgaatgatcgtaagtggtgttttgaaggccctgaggaacatgagatcttgaatgacagcggtgaaacagtgaagtgcagggctcctggaggagcaaagaagcctctgcgcccaaggtggtgtgatgaaagggtgtcatctgaccatagtgcgctgtctgaatttattaagtttgctgaaggtaggaggggagctgctgaagtgctagttgtgctgagtgaactccctgatttcctggttaaaaaaggtggagaggcaatggataccatcaatgtgttcctccactctgaggaaggctctagggcttaccgcaatgcactatcaatgatgcctgaggcaatgacaatagtcatgctgtttatactggctggactactgacatcgggaatggtcatctttttcatgtctcccaaaggcatcagtagaatgtctatggcgatgggcacaatggccggctgtggatatctcatgttccttggaggcgtcaaacccactcacatctcctatgtcatgctcatattctttgtcctgatggtggttgtgatccccgagccagggcaacaaaggtccatccaagacaaccaagtggcatacctcattattggcatcctgacgctggtttcagcggtggcagccaacgagctaggcatgctggagaaaaccaaagaggacctctttgggaagaagaacttaattccatctagtgcttcaccctggagttggccggatcttgacctgaagccaggagctgcctggacagtgtacgttggcattgttacaatgctctctccaatgttgcaccactggatcaaagtcgaatatggcaacctgtctctgtctggaatagcccagtcagcctcagtcctttctctcatggacaaggggataccattcatgaagatgaatatctcagtcataatgctgctggtcagtggctggaattcaataacagtgatgcctctgctctgtggcatagggtgcgccatgctccactggtctctcattttacctggaatcaaagcgcagcagtcaaggcttgcacagagaagggtgttccatggcgttgccaagaaccctgtggttgatgggaatccaacagttgacattgaggaagctcctgaaatgcctgccctttatgagaagaaactggctctatatctccttcttgctctcagcctagcttctgttgccatgtgcagaacgtccttttcattggctgaaggcattgtcctagcatcagctgccttagggccgctcatagagggaaacaccagccttctttggaatggacccatggctgtctccatgacaggagtcatgagggggaatcactatgcttttgtgggagtcatgtacaatctatggaagatgaaaactggacgccgggggagcgcgaatggaaaaactttgggtgaagtctggaagagggaactgaatctgttggacaagcgacagtttgagttgtataaaaggaccgacattgtggaggtggatcgtgatactgcacgcaggcatttggccgaagggaaggtggacaccggggtggcggtctccagggggaccgcaaagttaaggtggttccatgagcgtggctatgtcaagctggaaggtagggtgattgacctggggtgtggccgcggaggctggtgttactacgctgctgcgcaaaaggaagtgagtggggtcaaaggatttactcttggaagagacggccatgagaaacccatgaatgtgcaaagtctgggatggaacatcatcaccttcaaggacaaaactgatatccaccgcctggaaccagtgaaatgtgacacccttttgtgtgacattggagagtcatcatcgtcatcggtcacagagggggaaaggaccgtgagagttcttgatactgtagaaaaatggctggcttgtggggttgacaacttctgtgtgaaggtgttagctccatacatgccagatgttctcgagaaactggaattgctccaaaggaggtttggcggaacagtgatcaggaaccctctctccaggaattccactcatgaaatgtactacgtgtctggagcccgcagcaatgtcacatttactgtgaaccaaacatcccgcctcctgatgaggagaatgaggcgtccaactggaaaagtgaccctggaagctgacgtcatcctcccaattgggacacgcagtgttgagacagacaagggacccctggacaaagaggccatagaagaaagggttgagaggataaaatctgagtacatgacctcttggttttatgacaatgacaacccctacaggacctggcactactgtggctcctatgtcacaaaaacctcaggaagtgcggcgagcatggtaaatggtgttattaaaattctgacatatccatgggacaggatagaggaggtcacaagaatggcaatgactgacacaaccccttttggacagcaaagagtgtttaaagaaaaagttgacaccagagcaaaggatccaccagcgggaactaggaagatcatgaaagttgtcaacaggtggctgttccgccacctggccagagaaaagaaccctagactgtgcacaaaggaagaatttattgcaaaagtccgaagtcatgcagccattggagcttacctggaagaacaagaacagtggaagactgccaatgaggctgtccaagacccaaagttctgggaactggtggatgaagaaaggaagctgcaccaacaaggcaggtgtcggacttgtgtgtacaacatgatggggaaaagagagaagaagctgtcagagtttgggaaagcaaagggaagccgtgccatatggtatatgtggctgggagcgcggtatcttgagtttgaggccctgggattcctgaatgaggaccattgggcttccagggaaaactcaggaggaggagtggaaggcattggcttacaatacctaggatatgtgatcagagacctggctgcaatggatggtggtggattctacgcggatgacaccgctggatgggacacgcgcatcacagaggcagaccttgatgataacaggagatcttgatatacatgagcccacatcacaaaaaactggcacaagcagtgatggaaatgacatacaagaacaaagtggtgaaagtgttgagaccagccccaggagggaaagcctacatggatgtcataagtcgacgagaccagagaggatccgggcaggtagtgacttatgctctgaacaccatcaccaacttgaaagtccaattgatcagaatggcagaagcagagatggtgatacatcaccaacatgttcaagattgtgatgaatcagttctgaccaggctggaggcatggctcactgagcacggatgtgacagactgaagaggatggcggtgagtggagacgactgtgtggtccggcccatcgatgacaggttcggcctggccctgtcccatctcaacgccatgtccaaggttagaaaggacatatctgaatggcagccatcaaaagggtggaatgattgggagaatgtgcccttctgttcccaccacttccatgaactacagctgaaggatggcaggaggattgtggtgccttgccgagaacaggacgagctcattgggagaggaagggtgtctccaggaaacggctggatgatcaaggaaacagcttgcctcagcaaagcctatgccaacatgtggtcactgatgtattttcacaaaagggacatgaggctactgtcattggctgtttcctcagctgttcccacctcatgggttccacaaggacgcacaacatggtcgattcatgggaaaggggagtggatgaccacggaagacatgcttgaggtgtggaacagagtatggataaccaacaacccacacatgcaggacaagacaatggtgaaaaaatggagagatgtcccttatctaaccaagagacaagacaagctgtgcggatcactgattggaatgaccaatagggccacctgggcctcccacatccatttagtcatccatcgtatccgaacgctgattggacaggagaaatacactgactacctaacagtcatggacaggtattctgtggatgctgacctgcaactgggtgagcttatctgaaacaccatctaacaggaataaccgggatacaaaccacgggtggagaaccggactccccacaacctgaaaccgggatataaaccacggctggagaaccgggctccgcacttaaaatgaaacagaaaccgggataaaaactacggatggagaaccggactccacacattgagacagaagaagttgtcagcccagaacccaacacgagttttgccactgctaagctgtgaggcagtgcaggctgggacagccgacctccaggttgcgaaaaacctggtttctgggacctcccaccccagagtaaaaagaacggagcctccgctaccaccctcccacgtggtggtagaaagacggggtctagaggttagaggagaccctccagggaacaaatagtgggaccatattgacgccagggaaagaccggagtggttctctgcttttcctccagaggtctgtgagcacagtttgctcaagaataagcagacctttggatgacaaacacaaaaccact

SEQ ID NO: 10 - DNA, 36 bp, synthetic construct
  misc_feature 1..36: note = 5 UTR_For
  source 1..36: mol_type = other DNA
taatacgactcactataggagtaaatcctgtgtgct

SEQ ID NO: 11 - DNA, 30 bp, synthetic construct
  misc_feature 1..30: note = 5 UTR_Rev
  source 1..30: mol_type = other DNA
cagcatagggcattcatagctcatggtggc

SEQ ID NO: 12 - DNA, 30 bp, synthetic construct
  misc_feature 1..30: note = 3 UTR_For
  source 1..30: mol_type = other DNA
gtcatccatcgtatccgaacgctgattgga

SEQ ID NO: 13 - DNA, 30 bp, synthetic construct
  misc_feature 1..30: note = 3 UTR_Rev
  source 1..30: mol_type = other DNA
agtggttttgtgtttgtcatccaaaggtct

SEQ ID NO: 14 - DNA, 27 bp, synthetic construct
  misc_feature 1..27: note = NS5 region_For
  source 1..27: mol_type = other DNA
aaatgaaagtgcaacaatcttgatgac

SEQ ID NO: 15 - DNA, 26 bp, synthetic construct
  misc_feature 1..26: note = NS5 region_Rev
  source 1..26: mol_type = other DNA
tgttcaggaccaccacactctttcca

SEQ ID NO: 16 - DNA, 32 bp, synthetic construct
  misc_feature 1..32: note = cZik1-F
  source 1..32: mol_type = other DNA
agtaaatcctgtgtgctaattgaggtgcattg

SEQ ID NO: 17 - DNA, 25 bp, synthetic construct
  misc_feature 1..25: note = cZik1-R(2498)
  source 1..25: mol_type = other DNA
agcagagacggctgtggataagaag

SEQ ID NO: 18 - DNA, 32 bp, synthetic construct
  misc_feature 1..32: note = cZik2-F
  source 1..32: mol_type = other DNA
cagatggcggtggacatgcaaactctgacccc

SEQ ID NO: 19 - DNA, 32 bp, synthetic construct
  misc_feature 1..32: note = cZik2-R(5385)
  source 1..32: mol_type = other DNA
ctgccgtgagcggaaaaagcctgtgtgtggaa

SEQ ID NO: 20 - DNA, 32 bp, synthetic construct
  misc_feature 1..32: note = cZik3-F
  source 1..32: mol_type = other DNA
gaaatcggggctgtcgctcttgactatccgag

SEQ ID NO: 21 - DNA, 32 bp, synthetic construct
  misc_feature 1..32: note = cZik3-R(8205)
  source 1..32: mol_type = other DNA
ccacaagccagccatttttctacagtatcaag

SEQ ID NO: 22 - DNA, 32 bp, synthetic construct
  misc_feature 1..32: note = czika4-F
  source 1..32: mol_type = other DNA
caagctggaaggtagggtgattgacctggggt

SEQ ID NO: 23 - DNA, 32 bp, synthetic construct
  misc_feature 1..32: note = cZik4-R
  source 1..32: mol_type = other DNA
agtggttttgtgtttgtcatccaaaggtctgc

SEQ ID NO: 24 - DNA, 25 bp, synthetic construct
  misc_feature 1..25: note = cz-seq3
  source 1..25: mol_type = other DNA
caaaaaaggtgaagcacggagatct

SEQ ID NO: 25 - DNA, 26 bp, synthetic construct
  misc_feature 1..26: note = cz-seq4
  source 1..26: mol_type = other DNA
tggatgtggactttttggcaaaggga

SEQ ID NO: 26 - DNA, 27 bp, synthetic construct
  misc_feature 1..27: note = cz-seq5
  source 1..27: mol_type = other DNA
cagatggcggtggacatgcaaactctg

SEQ ID NO: 27 - DNA, 27 bp, synthetic construct
  misc_feature 1..27: note = cz-seq6
  source 1..27: mol_type = other DNA
agactctgatgactggctgaacaagta

SEQ ID NO: 28 - DNA, 29 bp, synthetic construct
  misc_feature 1..29: note = cz-seq7
  source 1..29: mol_type = other DNA
atgatccacaccttggaggcattagatta

SEQ ID NO: 29 - DNA, 30 bp, synthetic construct
  misc_feature 1..30: note = cz-seq8
  source 1..30: mol_type = other DNA
cgttgattgctgccttttcaatcagaccag

SEQ ID NO: 30 - DNA, 29 bp, synthetic construct
  misc_feature 1..29: note = cz-seq9
  source 1..29: mol_type = other DNA
ggttagcgtggctgggagggtggatgggc

SEQ ID NO: 31 - DNA, 30 bp, synthetic construct
  misc_feature 1..30: note = cz-seq10
  source 1..30: mol_type = other DNA
gaaatcggggctgtcgctcttgactatccg

SEQ ID NO: 32 - DNA, 27 bp, synthetic construct
  misc_feature 1..27: note = cz-seq11
  source 1..27: mol_type = other DNA
aaatgaaagtgcaacaatcttgatgac

SEQ ID NO: 33 - DNA, 28 bp, synthetic construct
  misc_feature 1..28: note = cz-seq12
  source 1..28: mol_type = other DNA
gatggagactcatactactattctgagc

SEQ ID NO: 34 - DNA, 28 bp, synthetic construct
  misc_feature 1..28: note = cz-seq13
  source 1..28: mol_type = other DNA
ctctagggcttaccgcaatgcactatca

SEQ ID NO: 35 - DNA, 29 bp, synthetic construct
  misc_feature 1..29: note = cz-seq14
  source 1..29: mol_type = other DNA
gtgatgcctctgctctgtggcatagggtg

SEQ ID NO: 36 - DNA, 29 bp, synthetic construct
  misc_feature 1..29: note = cz-seq15
  source 1..29: mol_type = other DNA
caagctggaaggtagggtgattgacctgg

SEQ ID NO: 37 - DNA, 27 bp, synthetic construct
  misc_feature 1..27: note = cz-seq16
  source 1..27: mol_type = other DNA
gagaggataaaatctgagtacatgacc

SEQ ID NO: 38 - DNA, 28 bp, synthetic construct
  misc_feature 1..28: note = cz-seq17
  source 1..28: mol_type = other DNA
cctggctgcaatggatggtggtggattc

SEQ ID NO: 39 - DNA, 30 bp, synthetic construct
  misc_feature 1..30: note = cz-seq18
  source 1..30: mol_type = other DNA
tgtgcccttctgttcccaccacttccatga

SEQ ID NO: 40 - DNA, 28 bp, synthetic construct
  misc_feature 1..28: note = cz-seq19
  source 1..28: mol_type = other DNA
gtggaacagagtatggataaccaacaac

SEQ ID NO: 41 - DNA, 29 bp, synthetic construct
  misc_feature 1..29: note = cz-seq20
  source 1..29: mol_type = other DNA
actccccacaacctgaaaccgggatataa